European Patent Application EP 4 779 020 A1, published July 22, 2026. Title: HYALURONIDASE OBTAINED FROM PURPUREOCILLIUM SP. AND ITS USE. Applicant: Consejo Superior de Investigaciones Científicas. Application EP. The sequence listing filed with the application follows.

SEQUENCE LISTING (21 sequences)

SEQ ID NO: 1 - protein, 378 aa, synthetic construct
APQRENAPTRTVEGDTAKRAVFKHPGIFVDSDRLKLMASKVAAAEQPWADAYSALKTHKYATRTKPTPYPTVECGPYSTPNVGCEDERADAMAAYANALMWAVTKDQAKADRAIEFMNAWAKTVKSHTNSNAPLQGAWAAADWARAGEIIRYTNAGWSSADITTFENMLRNVYLPLVKPGSQNPNNWELMFNEAAISISVFLNDKATYDSTMTRFLRSAAQYFYLKSDGPRPVKPAGMTDEKQDWWWNGQIARGLEDGIAMEICRDLTHTGYGIASVSHVIETSKIQGRDLYNEEVGTRLRYALEFQSKYDPKGGAVAAPSWLCDGTLKLHLEDVTEPGWNAMHHKYSMPWSGNFTLKHRPAGANTLFVGWETLTHAE

SEQ ID NO: 2 - protein, 399 aa, synthetic construct
MKLLTTLPALAAMMHLAVVHGAPQRENAPTRTVEGDTAKRAVFKHPGIFVDSDRLKLMASKVAAAEQPWADAYSALKTHKYATRTKPTPYPTVECGPYSTPNVGCEDERADAMAAYANALMWAVTKDQAKADRAIEFMNAWAKTVKSHTNSNAPLQGAWAAADWARAGEIIRYTNAGWSSADITTFENMLRNVYLPLVKPGSQNPNNWELMFNEAAISISVFLNDKATYDSTMTRFLRSAAQYFYLKSDGPRPVKPAGMTDEKQDWWWNGQIARGLEDGIAMEICRDLTHTGYGIASVSHVIETSKIQGRDLYNEEVGTRLRYALEFQSKYDPKGGAVAAPSWLCDGTLKLHLEDVTEPGWNAMHHKYSMPWSGNFTLKHRPAGANTLFVGWETLTHAE

SEQ ID NO: 3 - protein, 89 aa, synthetic construct
MRFPSIFTAVLFAASSALAAPVNTTTEDETAQIPAEAVIGYSDLEGDFDVAVLPFSNSTNNGLLFINTTIASIAAKEEGVSLEKREAEA

SEQ ID NO: 4 - protein, 467 aa, synthetic construct
MRFPSIFTAVLFAASSALAAPVNTTTEDETAQIPAEAVIGYSDLEGDFDVAVLPFSNSTNNGLLFINTTIASIAAKEEGVSLEKREAEAAPQRENAPTRTVEGDTAKRAVFKHPGIFVDSDRLKLMASKVAAAEQPWADAYSALKTHKYATRTKPTPYPTVECGPYSTPNVGCEDERADAMAAYANALMWAVTKDQAKADRAIEFMNAWAKTVKSHTNSNAPLQGAWAAADWARAGEIIRYTNAGWSSADITTFENMLRNVYLPLVKPGSQNPNNWELMFNEAAISISVFLNDKATYDSTMTRFLRSAAQYFYLKSDGPRPVKPAGMTDEKQDWWWNGQIARGLEDGIAMEICRDLTHTGYGIASVSHVIETSKIQGRDLYNEEVGTRLRYALEFQSKYDPKGGAVAAPSWLCDGTLKLHLEDVTEPGWNAMHHKYSMPWSGNFTLKHRPAGANTLFVGWETLTHAE

SEQ ID NO: 5 - DNA, 1137 bp, synthetic construct
  source 1..1137: mol_type = other DNA
gcaccacagcgggagaacgccccaacaaggactgttgaaggcgatactgccaagcgcgcagtcttcaaacaccccggcatttttgtcgattcagatcgcctcaagctcatggcgtccaaggtggccgccgcggagcagccgtgggccgatgcctacagcgcgctcaagactcacaagtacgccacgcggaccaagccgacgccgtacccgacggtcgagtgcggcccgtactcgacccctaacgtcggatgcgaggacgagagggccgacgccatggccgcgtacgccaacgccctcatgtgggccgtcaccaaggaccaggccaaggcggaccgggccatcgaattcatgaacgcctgggccaagacggtcaagtcgcacaccaactctaatgcgcctctgcagggcgcctgggcagccgcagactgggcgcgcgcgggcgagatcatccgctatacgaacgccggatggagcagtgccgacatcaccacctttgagaacatgttgcggaatgtctatctccctctggtcaagccagggtcccagaatcccaacaactgggagctgatgttcaacgaggcagctattagcatatccgtcttcctcaatgacaaagcaacgtacgactccaccatgacgcgcttcctcaggagcgcagcgcagtatttttatctcaagagcgacggcccgcgacctgtcaagcccgcaggcatgacggacgagaagcaggactggtggtggaatggccaaatcgcacgggggctcgaggacggcatcgccatggagatctgccgagacctcacccacacgggctacggcatcgcgtctgtctcgcacgtcattgagacgtccaagatccagggccgggacctgtacaacgaggaggtcggcactcggctgcggtacgcgctcgagttccagtccaagtacgatcccaagggcggagccgttgcagcgccgtcgtggctctgcgacgggacgctgaagctgcaccttgaggacgtcacggagccgggctggaatgccatgcaccacaagtacagcatgccgtggtctggcaacttcaccttgaagcacaggcctgccggcgccaacaccttgtttgttggttgggagacgctgacccatgctgagtga

SEQ ID NO: 6 - DNA, 1200 bp, synthetic construct
  source 1..1200: mol_type = other DNA
atgaagctcctcacaaccctaccggcccttgcggccatgatgcacctggcagtggtccacggcgcaccacagcgggagaacgccccaacaaggactgttgaaggcgatactgccaagcgcgcagtcttcaaacaccccggcatttttgtcgattcagatcgcctcaagctcatggcgtccaaggtggccgccgcggagcagccgtgggccgatgcctacagcgcgctcaagactcacaagtacgccacgcggaccaagccgacgccgtacccgacggtcgagtgcggcccgtactcgacccctaacgtcggatgcgaggacgagagggccgacgccatggccgcgtacgccaacgccctcatgtgggccgtcaccaaggaccaggccaaggcggaccgggccatcgaattcatgaacgcctgggccaagacggtcaagtcgcacaccaactctaatgcgcctctgcagggcgcctgggcagccgcagactgggcgcgcgcgggcgagatcatccgctatacgaacgccggatggagcagtgccgacatcaccacctttgagaacatgttgcggaatgtctatctccctctggtcaagccagggtcccagaatcccaacaactgggagctgatgttcaacgaggcagctattagcatatccgtcttcctcaatgacaaagcaacgtacgactccaccatgacgcgcttcctcaggagcgcagcgcagtatttttatctcaagagcgacggcccgcgacctgtcaagcccgcaggcatgacggacgagaagcaggactggtggtggaatggccaaatcgcacgggggctcgaggacggcatcgccatggagatctgccgagacctcacccacacgggctacggcatcgcgtctgtctcgcacgtcattgagacgtccaagatccagggccgggacctgtacaacgaggaggtcggcactcggctgcggtacgcgctcgagttccagtccaagtacgatcccaagggcggagccgttgcagcgccgtcgtggctctgcgacgggacgctgaagctgcaccttgaggacgtcacggagccgggctggaatgccatgcaccacaagtacagcatgccgtggtctggcaacttcaccttgaagcacaggcctgccggcgccaacaccttgtttgttggttgggagacgctgacccatgctgagtga

SEQ ID NO: 7 - DNA, 267 bp, synthetic construct
  source 1..267: mol_type = other DNA
atgagatttccttcaatttttactgctgttttattcgcagcatcctccgcattagctgctccagtcaacactacaacagaagatgaaacggcacaaattccggctgaagctgtcatcggttactcagatttagaaggggatttcgatgttgctgttttgccattttccaacagcacaaataacgggttattgtttataaatactactattgccagcattgctgctaaagaagaaggggtatctctcgagaaaagagaggctgaagct

SEQ ID NO: 8 - DNA, 1404 bp, synthetic construct
  source 1..1404: mol_type = other DNA
atgagatttccttcaatttttactgctgttttattcgcagcatcctccgcattagctgctccagtcaacactacaacagaagatgaaacggcacaaattccggctgaagctgtcatcggttactcagatttagaaggggatttcgatgttgctgttttgccattttccaacagcacaaataacgggttattgtttataaatactactattgccagcattgctgctaaagaagaaggggtatctctcgagaaaagagaggctgaagctgcaccacagcgggagaacgccccaacaaggactgttgaaggcgatactgccaagcgcgcagtcttcaaacaccccggcatttttgtcgattcagatcgcctcaagctcatggcgtccaaggtggccgccgcggagcagccgtgggccgatgcctacagcgcgctcaagactcacaagtacgccacgcggaccaagccgacgccgtacccgacggtcgagtgcggcccgtactcgacccctaacgtcggatgcgaggacgagagggccgacgccatggccgcgtacgccaacgccctcatgtgggccgtcaccaaggaccaggccaaggcggaccgggccatcgaattcatgaacgcctgggccaagacggtcaagtcgcacaccaactctaatgcgcctctgcagggcgcctgggcagccgcagactgggcgcgcgcgggcgagatcatccgctatacgaacgccggatggagcagtgccgacatcaccacctttgagaacatgttgcggaatgtctatctccctctggtcaagccagggtcccagaatcccaacaactgggagctgatgttcaacgaggcagctattagcatatccgtcttcctcaatgacaaagcaacgtacgactccaccatgacgcgcttcctcaggagcgcagcgcagtatttttatctcaagagcgacggcccgcgacctgtcaagcccgcaggcatgacggacgagaagcaggactggtggtggaatggccaaatcgcacgggggctcgaggacggcatcgccatggagatctgccgagacctcacccacacgggctacggcatcgcgtctgtctcgcacgtcattgagacgtccaagatccagggccgggacctgtacaacgaggaggtcggcactcggctgcggtacgcgctcgagttccagtccaagtacgatcccaagggcggagccgttgcagcgccgtcgtggctctgcgacgggacgctgaagctgcaccttgaggacgtcacggagccgggctggaatgccatgcaccacaagtacagcatgccgtggtctggcaacttcaccttgaagcacaggcctgccggcgccaacaccttgtttgttggttgggagacgctgacccatgctgagtga

SEQ ID NO: 9 - DNA, 1137 bp, synthetic construct
  source 1..1137: mol_type = other DNA
gctccacaaagagagaacgctccaactagaactgttgagggtgacactgctaagagagccgtttttaagcacccaggtatcttcgttgactccgacagattgaagttgatggcttccaaggttgctgctgctgaacaaccatgggctgatgcttactccgctcttaagactcacaagtacgccaccagaactaagccaactccatatccaaccgttgagtgtggtccatactccactccaaacgttggttgtgaagatgaacgtgctgatgctatggctgcttacgctaacgctttgatgtgggctgttactaaggaccaagctaaggctgacagagccatcgaattcatgaacgcttgggctaagactgtcaagtcccacactaactctaacgccccattgcaaggtgcttgggctgctgcagattgggctagagctggtgagattatcagatacactaacgctggttggtcctccgctgacattactactttcgagaacatgctgaggaacgtctacttgccattggtcaagccaggttctcagaacccaaacaactgggagttgatgttcaacgaggctgctatttccatctccgtgttcttgaacgacaaggctacttacgactccaccatgaccagattcttgagatccgctgctcagtacttctacttgaagtctgacggtccaagaccagttaagccagctggtatgactgacgaaaagcaagattggtggtggaacggtcagatcgctagaggtttggaagatggtatcgccatggaaatctgcagagacttgactcacactggttacggtatcgcttctgtttcccacgttatcgagacttccaagatccagggtagagacttgtacaacgaagaggtcggtactagattgagatacgccttggagttccagtccaagtacgatccaaaaggtggtgctgttgctgctccatcttggttgtgtgatggtactttgaagctgcacttggaggacgttactgaaccaggttggaacgctatgcaccacaagtactctatgccatggtccggtaacttcaccttgaagcacagacctgctggtgctaacactttgttcgttggttgggaaactttgacccacgctgagtaa

SEQ ID NO: 10 - DNA, 1200 bp, synthetic construct
  source 1..1200: mol_type = other DNA
atgaagttgctgactaccttgccagctttggctgctatgatgcacttggctgttgttcatggtgctccacaaagagagaacgctccaactagaactgttgagggtgacactgctaagagagccgtttttaagcacccaggtatcttcgttgactccgacagattgaagttgatggcttccaaggttgctgctgctgaacaaccatgggctgatgcttactccgctcttaagactcacaagtacgccaccagaactaagccaactccatatccaaccgttgagtgtggtccatactccactccaaacgttggttgtgaagatgaacgtgctgatgctatggctgcttacgctaacgctttgatgtgggctgttactaaggaccaagctaaggctgacagagccatcgaattcatgaacgcttgggctaagactgtcaagtcccacactaactctaacgccccattgcaaggtgcttgggctgctgcagattgggctagagctggtgagattatcagatacactaacgctggttggtcctccgctgacattactactttcgagaacatgctgaggaacgtctacttgccattggtcaagccaggttctcagaacccaaacaactgggagttgatgttcaacgaggctgctatttccatctccgtgttcttgaacgacaaggctacttacgactccaccatgaccagattcttgagatccgctgctcagtacttctacttgaagtctgacggtccaagaccagttaagccagctggtatgactgacgaaaagcaagattggtggtggaacggtcagatcgctagaggtttggaagatggtatcgccatggaaatctgcagagacttgactcacactggttacggtatcgcttctgtttcccacgttatcgagacttccaagatccagggtagagacttgtacaacgaagaggtcggtactagattgagatacgccttggagttccagtccaagtacgatccaaaaggtggtgctgttgctgctccatcttggttgtgtgatggtactttgaagctgcacttggaggacgttactgaaccaggttggaacgctatgcaccacaagtactctatgccatggtccggtaacttcaccttgaagcacagacctgctggtgctaacactttgttcgttggttgggaaactttgacccacgctgagtaa

SEQ ID NO: 11 - DNA, 1404 bp, synthetic construct
  source 1..1404: mol_type = other DNA
atgagatttccttcaatttttactgctgttttattcgcagcatcctccgcattagctgctccagtcaacactacaacagaagatgaaacggcacaaattccggctgaagctgtcatcggttactcagatttagaaggggatttcgatgttgctgttttgccattttccaacagcacaaataacgggttattgtttataaatactactattgccagcattgctgctaaagaagaaggggtatctctcgagaaaagagaggctgaagctgctccacaaagagagaacgctccaactagaactgttgagggtgacactgctaagagagccgtttttaagcacccaggtatcttcgttgactccgacagattgaagttgatggcttccaaggttgctgctgctgaacaaccatgggctgatgcttactccgctcttaagactcacaagtacgccaccagaactaagccaactccatatccaaccgttgagtgtggtccatactccactccaaacgttggttgtgaagatgaacgtgctgatgctatggctgcttacgctaacgctttgatgtgggctgttactaaggaccaagctaaggctgacagagccatcgaattcatgaacgcttgggctaagactgtcaagtcccacactaactctaacgccccattgcaaggtgcttgggctgctgcagattgggctagagctggtgagattatcagatacactaacgctggttggtcctccgctgacattactactttcgagaacatgctgaggaacgtctacttgccattggtcaagccaggttctcagaacccaaacaactgggagttgatgttcaacgaggctgctatttccatctccgtgttcttgaacgacaaggctacttacgactccaccatgaccagattcttgagatccgctgctcagtacttctacttgaagtctgacggtccaagaccagttaagccagctggtatgactgacgaaaagcaagattggtggtggaacggtcagatcgctagaggtttggaagatggtatcgccatggaaatctgcagagacttgactcacactggttacggtatcgcttctgtttcccacgttatcgagacttccaagatccagggtagagacttgtacaacgaagaggtcggtactagattgagatacgccttggagttccagtccaagtacgatccaaaaggtggtgctgttgctgctccatcttggttgtgtgatggtactttgaagctgcacttggaggacgttactgaaccaggttggaacgctatgcaccacaagtactctatgccatggtccggtaacttcaccttgaagcacagacctgctggtgctaacactttgttcgttggttgggaaactttgacccacgctgagtaa

SEQ ID NO: 12 - DNA, 26 bp, synthetic construct
  source 1..26: mol_type = other DNA
atgaagttgctgactaccttgccagc

SEQ ID NO: 13 - DNA, 25 bp, synthetic construct
  source 1..25: mol_type = other DNA
ttactcagcgtgggtcaaagtttcc

SEQ ID NO: 14 - DNA, 19 bp, synthetic construct
  source 1..19: mol_type = other DNA
gaattcgagctcggtaccc

SEQ ID NO: 15 - DNA, 21 bp, synthetic construct
  source 1..21: mol_type = other DNA
agcttcagcctctcttttctc

SEQ ID NO: 16 - DNA, 53 bp, synthetic construct
  source 1..53: mol_type = other DNA
ggtatctctcgagaaaagagaggctgaagctgctccacaaagagagaacgctc

SEQ ID NO: 17 - DNA, 49 bp, synthetic construct
  source 1..49: mol_type = other DNA
atccccgggtaccgagctcgaattcttactcagcgtgggtcaaagtttc

SEQ ID NO: 18 - DNA, 21 bp, synthetic construct
  source 1..21: mol_type = other DNA
gactggttccaattgacaagc

SEQ ID NO: 19 - DNA, 21 bp, synthetic construct
  source 1..21: mol_type = other DNA
gcaaatggcattctgacatcc

SEQ ID NO: 20 - DNA, 19 bp, synthetic construct
  source 1..19: mol_type = other DNA
taatacgactcactatagg

SEQ ID NO: 21 - DNA, 19 bp, synthetic construct
  source 1..19: mol_type = other DNA
atttaggtgacactataga